European Patent Application EP 4 707 305 A1, published March 11, 2026. Title: 抗CLDN6抗体及其用途. Applicant: 智泽童康（广州）生物科技有限公司. The sequence listing filed with the application follows.

SEQUENCE LISTING (179 sequences)

SEQ ID NO: 1 - protein, 5 aa, synthetic construct
SYNIH

SEQ ID NO: 2 - protein, 5 aa, synthetic construct
SYGMS

SEQ ID NO: 3 - protein, 5 aa, synthetic construct
NYAMS

SEQ ID NO: 4 - protein, 5 aa, synthetic construct
SYGIS

SEQ ID NO: 5 - protein, 5 aa, synthetic construct
DYNMH

SEQ ID NO: 6 - protein, 8 aa, synthetic construct
GYSFTGYT

SEQ ID NO: 7 - protein, 5 aa, synthetic construct
SYNMH

SEQ ID NO: 8 - protein, 17 aa, synthetic construct
YIYPGNGGTKYNERFKG

SEQ ID NO: 9 - protein, 17 aa, synthetic construct
TISSGGSYTYYPDSVKG

SEQ ID NO: 10 - protein, 17 aa, synthetic construct
TISDGGSYTSYPDNIKG

SEQ ID NO: 11 - protein, 17 aa, synthetic construct
EIYPRSGNTYHNEKFKG

SEQ ID NO: 12 - protein, 17 aa, synthetic construct
YVNPNNGATSYNQKFKG

SEQ ID NO: 13 - protein, 17 aa, synthetic construct
YINPNNGATNYNQKFKG

SEQ ID NO: 14 - protein, 9 aa, synthetic construct
INPYNGGTI

SEQ ID NO: 15 - protein, 17 aa, synthetic construct
YIYPGNGGTNYNQKFKG

SEQ ID NO: 16 - protein, 14 aa, synthetic construct
WRYYDRPTHYAMDY

SEQ ID NO: 17 - protein, 11 aa, synthetic construct
PHYVSSYAMDY

SEQ ID NO: 18 - protein, 12 aa, synthetic construct
DAILITTAGFAY

SEQ ID NO: 19 - protein, 10 aa, synthetic construct
SSYDYYAMDY

SEQ ID NO: 20 - protein, 12 aa, synthetic construct
WDGYVYYYGLDY

SEQ ID NO: 21 - protein, 12 aa, synthetic construct
WDGYVYYYGMDY

SEQ ID NO: 22 - protein, 10 aa, synthetic construct
ARDYGFVLDY

SEQ ID NO: 23 - protein, 14 aa, synthetic construct
WKYYDKTTHYALDY

SEQ ID NO: 24 - protein, 15 aa, synthetic construct
RASKSVSTSGFSYLH

SEQ ID NO: 25 - protein, 11 aa, synthetic construct
KASEDIYNRLA

SEQ ID NO: 26 - protein, 12 aa, synthetic construct
SVSSIISSSKLH

SEQ ID NO: 27 - protein, 11 aa, synthetic construct
KASDHINNWLA

SEQ ID NO: 28 - protein, 5 aa, synthetic construct
SSVSY

SEQ ID NO: 29 - protein, 15 aa, synthetic construct
RASKSVSTSGYSYIH

SEQ ID NO: 30 - protein, 7 aa, synthetic construct
LASNLES

SEQ ID NO: 31 - protein, 7 aa, synthetic construct
GATSLET

SEQ ID NO: 32 - protein, 7 aa, synthetic construct
ATTSLET

SEQ ID NO: 33 - protein, 7 aa, synthetic construct
GTSNLAS

SEQ ID NO: 34 - protein, 9 aa, synthetic construct
QHSREFPFT

SEQ ID NO: 35 - protein, 9 aa, synthetic construct
QQYWSTPPT

SEQ ID NO: 36 - protein, 9 aa, synthetic construct
QQYWSFPRT

SEQ ID NO: 37 - protein, 9 aa, synthetic construct
QQYWSTPYT

SEQ ID NO: 38 - protein, 9 aa, synthetic construct
QQYWNTPYT

SEQ ID NO: 39 - protein, 10 aa, synthetic construct
QQRSIYPPWT

SEQ ID NO: 40 - protein, 9 aa, synthetic construct
HHSRELPFT

SEQ ID NO: 41 - protein, 123 aa, synthetic construct
QAYLQQSGAELVRSGASVKMSCKASGYTFTSYNIHWVKQTPGQGLEWIGYIYPGNGGTKYNERFKGKATLTADASSSTAYMQISSLTSEDSAVYFCARWRYYDRPTHYAMDYWGQGTSVTVSS

SEQ ID NO: 42 - protein, 120 aa, synthetic construct
EVQLVESGGDLVKPGGSLKLSCAASGFTFSSYGMSWVRQTPDKRLEWVATISSGGSYTYYPDSVKGRFTISRDNAKNTLYLQMSSLKSEDTAMYYCARPHYVSSYAMDYWGQGTSVTVSS

SEQ ID NO: 43 - protein, 121 aa, synthetic construct
EVQLVESGGGLVKPGGSLKLSCAASGFTFSNYAMSWVRQTPEKRLEWVATISDGGSYTSYPDNIKGRFTISRDNAKNNLYLQVTHLKSEDTAMYYCARDAILITTAGFAYWGQGTLLTVSA

SEQ ID NO: 44 - protein, 119 aa, synthetic construct
QGQLQQSGAELARPGASVKLSCKASGYTFTSYGISWVKQRTGQGLEWIGEIYPRSGNTYHNEKFKGKATLTADKSSSTAYMELRSLTSEDSAVYFCARSSYDYYAMDYWGQGTSVTVSS

SEQ ID NO: 45 - protein, 121 aa, synthetic construct
EVQLQQSGPELVKPGASVKMSCKASGYTFTDYNMHWVKKSHGKSLEWIGYVNPNNGATSYNQKFKGKATLTVNKSSSTAYMELRSLTSEDSAVYNCARWDGYVYYYGLDYWGQGTSVTVSS

SEQ ID NO: 46 - protein, 121 aa, synthetic construct
EVQLQQSGPELVKPGASVKMSCKASGYTFTDYNMHWVKKSHGKSLEWIGYINPNNGATNYNQKFKGKATLTVNKSSSTAYMELRSLTSEDSAVYNCARWDGYVYYYGMDYWGQGTSVTVSS

SEQ ID NO: 47 - protein, 117 aa, synthetic construct
EVQLQQSGPELVKPGASMKISCKASGYSFTGYTMNWVKQSHGKNLEWIGLINPYNGGTIYNQKFKGKATLTVDKSSSTAYMELLSLTSEDSAVYYCARDYGFVLDYWGQGTTLTVSS

SEQ ID NO: 48 - protein, 123 aa, synthetic construct
QAYLQQSGAELVRSGASVKMSCKASGYTFTSYNMHWVKQTPGQGLEWIGYIYPGNGGTNYNQKFKGKATLTADTSSSTAYMQISSLTSEDSAVYFCARWKYYDKTTHYALDYWGQGTLVTVSS

SEQ ID NO: 49 - protein, 121 aa, synthetic construct
QVQLVQSGAEVKKPGASVKVSCKASGYTFTDYNMHWVRQAPGQGLEWIGYVNPNNGATSYNQKFKGRATMTRDTSTSTVYMELSSLRSEDTAVYYCARWDGYVYYYGLDYWGQGTLVTVSS

SEQ ID NO: 50 - protein, 121 aa, synthetic construct
QVQLVQSGAEVKKPGASVKVSCKASGYTFTDYNMHWVRQAPGQGLEWIGYVNPNNGATSYNQKFKGRVTMTVDTSTSTVYMELSSLRSEDTAVYNCARWDGYVYYYGLDYWGQGTLVTVSS

SEQ ID NO: 51 - protein, 121 aa, synthetic construct
QVQLVQSGAEVKKPGASVKVSCKASGYTFTDYNMHWVRQAPGQGLEWIGYVNPNNGATSYNQKFKGRATMTVDTSTSTVYMELSSLRSEDTAVYNCARWDGYVYYYGLDYWGQGTLVTVSS

SEQ ID NO: 52 - protein, 121 aa, synthetic construct
QVQLVQSGAEVKKPGASVKVSCKASGYTFTDYNMHWVRQAPGQSLEWIGYVNPNNGATSYNQKFKGRATMTVDKSTSTVYMELSSLRSEDTAVYNCARWDGYVYYYGLDYWGQGTLVTVSS

SEQ ID NO: 53 - protein, 121 aa, synthetic construct
QVQLVQSGAEVKKPGASVKVSCKASGYTFTDYNMHWVRQAPGQRLEWIGYINPNNGATNYNQKFKGRATITVDTSASTAYMELSSLRSEDTAVYYCARWDGYVYYYGMDYWGQGTLVTVSS

SEQ ID NO: 54 - protein, 121 aa, synthetic construct
QVQLVQSGAEVKKPGASVKVSCKASGYTFTDYNMHWVRQAPGQSLEWIGYINPNNGATNYNQKFKGRATITVDKSASTAYMELSSLRSEDTAVYNCARWDGYVYYYGMDYWGQGTLVTVSS

SEQ ID NO: 55 - protein, 121 aa, synthetic construct
QVQLVQSGAEVKKPGASVKVSCKASGYTFTDYNMHWVRQAPGQRLEWIGYINPNNGATNYNQKFKGRVTITVDTSASTAYMELSSLRSEDTAVYNCARWDGYVYYYGMDYWGQGTLVTVSS

SEQ ID NO: 56 - protein, 121 aa, synthetic construct
QVQLVQSGAEVKKPGASVKVSCKASGYTFTDYNMHWVRQAPGQSLEWIGYINPNNGATNYNQKFKGRATITVDTSASTAYMELSSLRSEDTAVYNCARWDGYVYYYGMDYWGQGTLVTVSS

SEQ ID NO: 57 - protein, 121 aa, synthetic construct
QVQLVQSGAEVKKPGASVKVSCKASGYTFTDYNMHWVRQATGQGLEWIGYINPNNGATNYNQKFKGRATMTRNKSISTAYMELRSLRSEDTAVYYCARWDGYVYYYGMDYWGQGTLVTVSS

SEQ ID NO: 58 - protein, 121 aa, synthetic construct
QVQLVQSGAEVKKPGASVKVSCKASGYTFTDYNMHWVRQATGQGLEWIGYINPNNGATNYNQKFKGRATMTRNKSISTAYMELRSLRSEDTAVYNCARWDGYVYYYGMDYWGQGTLVTVSS

SEQ ID NO: 59 - protein, 121 aa, synthetic construct
QVQLVQSGAEVKKPGASVKVSCKASGYTFTDYNMHWVRQATGQGLEWIGYINPNNGATNYNQKFKGRATLTVNKSISTAYMELRSLRSEDTAVYYCARWDGYVYYYGMDYWGQGTLVTVSS

SEQ ID NO: 60 - protein, 121 aa, synthetic construct
QVQLVQSGAEVKKPGASVKVSCKASGYTFTDYNMHWVRKATGQSLEWIGYINPNNGATNYNQKFKGRATMTRNKSISTAYMELRSLRSEDTAVYNCARWDGYVYYYGMDYWGQGTLVTVSS

SEQ ID NO: 61 - protein, 111 aa, synthetic construct
DIVVTQSPASLAVSLGQRATISCRASKSVSTSGFSYLHWFQQKPGQPPKLLIYLASNLESGVPARFSGSGSGTDFTLNIHPVEEEDVAVYYCQHSREFPFTFGSGTKLEIK

SEQ ID NO: 62 - protein, 107 aa, synthetic construct
DIQMTQSSSSFSVSLGDRVTITCKASEDIYNRLAWYQQKPGNAPRLLISGATSLETGVPSRFSGSGSGKDYTLSITSLQTEDVATYYCQQYWSTPPTFGGGTKLEIK

SEQ ID NO: 63 - protein, 107 aa, synthetic construct
DIQMTQSSSSFSVSLGDRVTITCKASEDIYNRLAWYQQKPGNAPRLLISATTSLETGVPSRFSGSGSGKDYTLSITSLQTEDVATYYCQQYWSFPRTFGGGTKLEVK

SEQ ID NO: 64 - protein, 108 aa, synthetic construct
EIVVTQSPALMAASPGEKVTITCSVSSIISSSKLHWYQQKSETSPKPWIYGTSNLASGVPIRFSGSGSGTSYSLTISSMEAEDAATYYCQQWSSYPLTFGAGTKLELK

SEQ ID NO: 65 - protein, 107 aa, synthetic construct
DIQMTQSSSYLSVSLGGRVTITCKASDHINNWLAWYQQKPGNAPRLLISGATSLETGVPSRFSGSGSGKDYTLSITSLQTEDVATYYCQQYWSTPYTFGGGTKLEIK

SEQ ID NO: 66 - protein, 107 aa, synthetic construct
DIQMTQSSSYLSVSLGGRVTITCKASDHINNWLAWYQQKPGNAPRLLISGATSLETGVPSRFSGSGSGKDYTLSITSLQTEDVATYYCQQYWNTPYTFGGGTKLEIK

SEQ ID NO: 67 - protein, 106 aa, synthetic construct
IVLTQSPAIMSASPGEKVTITCSASSSVSYLHWFQQKPGTSPKLWVYSTSNLPSGVPARFGGSGSGTSYSLTISRMEAEDAATYYCQQRSIYPPWTFGGGTKLEIK

SEQ ID NO: 68 - protein, 111 aa, synthetic construct
DIVLTQSPASLAVSLGQWATISCRASKSVSTSGYSYIHWHQQKPGQPPKLLIYLASNLESGVPARFSGSGSGTDFTLNIHPVEEEDAATYYCHHSRELPFTFGSGTKLEIK

SEQ ID NO: 69 - protein, 107 aa, synthetic construct
DIQMTQSPSSLSASVGDRVTITCKASDHINNWLAWYQQKPGKVPKLLISGATSLETGVPSRFSGSGSGTDYTLTISSLQPEDVATYYCQQYWSTPYTFGGGTKLEIK

SEQ ID NO: 70 - protein, 107 aa, synthetic construct
DIQMTQSPSSLSASVGGRVTITCKASDHINNWLAWYQQKPGKVPRLLISGATSLETGVPSRFSGSGSGTDYTLTISSLQPEDVATYYCQQYWSTPYTFGGGTKLEIK

SEQ ID NO: 71 - protein, 107 aa, synthetic construct
DIQMTQSPSSLSASVGDRVTITCKASDHINNWLAWYQQKPGKAPKLLISGATSLETGVPSRFSGSGSGTDYTFTISSLQPEDIATYYCQQYWNTPYTFGGGTKLEIK

SEQ ID NO: 72 - protein, 107 aa, synthetic construct
DIQMTQSPSSLSASVGGRVTITCKASDHINNWLAWYQQKPGKAPKLLISGATSLETGVPSRFSGSGSGTDYTFTISSLQPEDIATYYCQQYWNTPYTFGGGTKLEIK

SEQ ID NO: 73 - protein, 107 aa, synthetic construct
DIQMTQSPSSLSASVGDRVTITCKASDHINNWLAWYQQKPGKVPRLLISGATSLETGVPSRFSGSGSGKDYTLTISSLQPEDVATYYCQQYWNTPYTFGGGTKLEIK

SEQ ID NO: 74 - protein, 17 aa, synthetic construct
YIYPGNAGTNYNQKFKG

SEQ ID NO: 75 - protein, 17 aa, synthetic construct
YVNPNNAATSYNQKFKG

SEQ ID NO: 76 - protein, 17 aa, synthetic construct
YVNPNQGATSYNQKFKG

SEQ ID NO: 77 - protein, 12 aa, synthetic construct
WDAYVYYYGLDY

SEQ ID NO: 78 - protein, 12 aa, synthetic construct
WEGYVYYYGLDY

SEQ ID NO: 79 - protein, 123 aa, synthetic construct
QAYLQQSGAELVRSGASVKMSCKASGYTFTSYNMHWVKQTPGQGLEWIGYIYPGNAGTNYNQKFKGKATLTADTSSSTAYMQISSLTSEDSAVYFCARWKYYDKTTHYALDYWGQGTLVTVSS

SEQ ID NO: 80 - protein, 121 aa, synthetic construct
EVQLQQSGPELVKPGASVKMSCKASGYTFTDYNMHWVKKSHGKSLEWIGYVNPNNAATSYNQKFKGKATLTVNKSSSTAYMELRSLTSEDSAVYNCARWDGYVYYYGLDYWGQGTSVTVSS

SEQ ID NO: 81 - protein, 121 aa, synthetic construct
EVQLQQSGPELVKPGASVKMSCKASGYTFTDYNMHWVKKSHGKSLEWIGYVNPNQGATSYNQKFKGKATLTVNKSSSTAYMELRSLTSEDSAVYNCARWDGYVYYYGLDYWGQGTSVTVSS

SEQ ID NO: 82 - protein, 121 aa, synthetic construct
EVQLQQSGPELVKPGASVKMSCKASGYTFTDYNMHWVKKSHGKSLEWIGYVNPNNGATSYNQKFKGKATLTVNKSSSTAYMELRSLTSEDSAVYNCARWDAYVYYYGLDYWGQGTSVTVSS

SEQ ID NO: 83 - protein, 121 aa, synthetic construct
EVQLQQSGPELVKPGASVKMSCKASGYTFTDYNMHWVKKSHGKSLEWIGYVNPNNGATSYNQKFKGKATLTVNKSSSTAYMELRSLTSEDSAVYNCARWEGYVYYYGLDYWGQGTSVTVSS

SEQ ID NO: 84 - protein, 330 aa, synthetic construct [sequence omitted]

SEQ ID NO: 85 - protein, 107 aa, synthetic construct [sequence omitted]

SEQ ID NO: 86 - protein, 19 aa, synthetic construct
MGWSCIILFLVATATGVHS

SEQ ID NO: 87 - protein, 451 aa, synthetic construct
EVQLQQSGPELVKPGASVKMSCKASGYTFTDYNMHWVKKSHGKSLEWIGYVNPNNGATSYNQKFKGKATLTVNKSSSTAYMELRSLTSEDSAVYNCARWDGYVYYYGLDYWGQGTSVTVSSASTKGPSVFPLAPSSKSTSGGTAALGCLVKDYFPEPVTVSWNSGALTSGVHTFPAVLQSSGLYSLSSVVTVPSSSLGTQTYICNVNHKPSNTKVDKKVEPKSCDKTHTCPPCPAPELLGGPSVFLFPPKPKDTLMISRTPEVTCVVVDVSHEDPEVKFNWYVDGVEVHNAKTKPREEQYNSTYRVVSVLTVLHQDWLNGKEYKCKVSNKALPAPIEKTISKAKGQPREPQVYTLPPSRDELTKNQVSLTCLVKGFYPSDIAVEWESNGQPENNYKTTPPVLDSDGSFFLYSKLTVDKSRWQQGNVFSCSVMHEALHNHYTQKSLSLSPGK

SEQ ID NO: 88 - protein, 214 aa, synthetic construct
DIQMTQSSSYLSVSLGGRVTITCKASDHINNWLAWYQQKPGNAPRLLISGATSLETGVPSRFSGSGSGKDYTLSITSLQTEDVATYYCQQYWSTPYTFGGGTKLEIKRTVAAPSVFIFPPSDEQLKSGTASVVCLLNNFYPREAKVQWKVDNALQSGNSQESVTEQDSKDSTYSLSSTLTLSKADYEKHKVYACEVTHQGLSSPVTKSFNRGEC

SEQ ID NO: 89 - protein, 470 aa, synthetic construct
MGWSCIILFLVATATGVHSEVQLQQSGPELVKPGASVKMSCKASGYTFTDYNMHWVKKSHGKSLEWIGYVNPNNGATSYNQKFKGKATLTVNKSSSTAYMELRSLTSEDSAVYNCARWDGYVYYYGLDYWGQGTSVTVSSASTKGPSVFPLAPSSKSTSGGTAALGCLVKDYFPEPVTVSWNSGALTSGVHTFPAVLQSSGLYSLSSVVTVPSSSLGTQTYICNVNHKPSNTKVDKKVEPKSCDKTHTCPPCPAPELLGGPSVFLFPPKPKDTLMISRTPEVTCVVVDVSHEDPEVKFNWYVDGVEVHNAKTKPREEQYNSTYRVVSVLTVLHQDWLNGKEYKCKVSNKALPAPIEKTISKAKGQPREPQVYTLPPSRDELTKNQVSLTCLVKGFYPSDIAVEWESNGQPENNYKTTPPVLDSDGSFFLYSKLTVDKSRWQQGNVFSCSVMHEALHNHYTQKSLSLSPGK

SEQ ID NO: 90 - protein, 233 aa, synthetic construct
MGWSCIILFLVATATGVHSDIQMTQSSSYLSVSLGGRVTITCKASDHINNWLAWYQQKPGNAPRLLISGATSLETGVPSRFSGSGSGKDYTLSITSLQTEDVATYYCQQYWSTPYTFGGGTKLEIKRTVAAPSVFIFPPSDEQLKSGTASVVCLLNNFYPREAKVQWKVDNALQSGNSQESVTEQDSKDSTYSLSSTLTLSKADYEKHKVYACEVTHQGLSSPVTKSFNRGEC

SEQ ID NO: 91 - protein, 17 aa, synthetic construct
YANPNNGATSYNQKFKG

SEQ ID NO: 92 - protein, 17 aa, synthetic construct
YINPNNGATSYNQKFKG

SEQ ID NO: 93 - protein, 17 aa, synthetic construct
YLNPNNGATSYNQKFKG

SEQ ID NO: 94 - protein, 17 aa, synthetic construct
YVNPNNGASSYNQKFKG

SEQ ID NO: 95 - protein, 12 aa, synthetic construct
WDGYVYYYGVDY

SEQ ID NO: 96 - protein, 12 aa, synthetic construct
WDGYVYYYGLDF

SEQ ID NO: 97 - protein, 12 aa, synthetic construct
WDGYSYYYGLDY

SEQ ID NO: 98 - protein, 11 aa, synthetic construct
KASEHINNWLA

SEQ ID NO: 99 - protein, 11 aa, synthetic construct
KASDHVNNWLA

SEQ ID NO: 100 - protein, 11 aa, synthetic construct
KASDHINQWLA

SEQ ID NO: 101 - protein, 7 aa, synthetic construct
GGTSLET

SEQ ID NO: 102 - protein, 9 aa, synthetic construct
QQYWSTPYS

SEQ ID NO: 103 - protein, 9 aa, synthetic construct
QQYGSTPYT

SEQ ID NO: 104 - protein, 9 aa, synthetic construct
QQYWHTPYT

SEQ ID NO: 105 - protein, 121 aa, synthetic construct
QVQLVQSGAEVKKPGASVKVSCKASGYTFTDYNMHWVRQAPGQSLEWIGYANPNNGATSYNQKFKGRATMTVDKSTSTVYMELSSLRSEDTAVYNCARWDGYVYYYGLDYWGQGTLVTVSS

SEQ ID NO: 106 - protein, 121 aa, synthetic construct
QVQLVQSGAEVKKPGASVKVSCKASGYTFTDYNMHWVRQAPGQSLEWIGYINPNNGATSYNQKFKGRATMTVDKSTSTVYMELSSLRSEDTAVYNCARWDGYVYYYGLDYWGQGTLVTVSS

SEQ ID NO: 107 - protein, 121 aa, synthetic construct
QVQLVQSGAEVKKPGASVKVSCKASGYTFTDYNMHWVRQAPGQSLEWIGYLNPNNGATSYNQKFKGRATMTVDKSTSTVYMELSSLRSEDTAVYNCARWDGYVYYYGLDYWGQGTLVTVSS

SEQ ID NO: 108 - protein, 121 aa, synthetic construct
QVQLVQSGAEVKKPGASVKVSCKASGYTFTDYNMHWVRQAPGQSLEWIGYVNPNNGASSYNQKFKGRATMTVDKSTSTVYMELSSLRSEDTAVYNCARWDGYVYYYGLDYWGQGTLVTVSS

SEQ ID NO: 109 - protein, 121 aa, synthetic construct
QVQLVQSGAEVKKPGASVKVSCKASGYTFTDYNMHWVRQAPGQSLEWIGYVNPNNGATSYNQKFKGRATMTVDKSTSTVYMELSSLRSEDTAVYNCARWDGYVYYYGVDYWGQGTLVTVSS

SEQ ID NO: 110 - protein, 121 aa, synthetic construct
QVQLVQSGAEVKKPGASVKVSCKASGYTFTDYNMHWVRQAPGQSLEWIGYVNPNNGATSYNQKFKGRATMTVDKSTSTVYMELSSLRSEDTAVYNCARWDGYVYYYGLDFWGQGTLVTVSS

SEQ ID NO: 111 - protein, 121 aa, synthetic construct
QVQLVQSGAEVKKPGASVKVSCKASGYTFTDYNMHWVRQAPGQSLEWIGYVNPNNGATSYNQKFKGRATMTVDKSTSTVYMELSSLRSEDTAVYNCARWDGYSYYYGLDYWGQGTLVTVSS

SEQ ID NO: 112 - protein, 107 aa, synthetic construct
DIQMTQSPSSLSASVGDRVTITCKASEHINNWLAWYQQKPGKVPKLLISGATSLETGVPSRFSGSGSGTDYTLTISSLQPEDVATYYCQQYWSTPYTFGGGTKLEIK

SEQ ID NO: 113 - protein, 107 aa, synthetic construct
DIQMTQSPSSLSASVGDRVTITCKASDHVNNWLAWYQQKPGKVPKLLISGATSLETGVPSRFSGSGSGTDYTLTISSLQPEDVATYYCQQYWSTPYTFGGGTKLEIK

SEQ ID NO: 114 - protein, 107 aa, synthetic construct
DIQMTQSPSSLSASVGDRVTITCKASDHINQWLAWYQQKPGKVPKLLISGATSLETGVPSRFSGSGSGTDYTLTISSLQPEDVATYYCQQYWSTPYTFGGGTKLEIK

SEQ ID NO: 115 - protein, 107 aa, synthetic construct
DIQMTQSPSSLSASVGDRVTITCKASDHINNWLAWYQQKPGKVPKLLISGGTSLETGVPSRFSGSGSGTDYTLTISSLQPEDVATYYCQQYWSTPYTFGGGTKLEIK

SEQ ID NO: 116 - protein, 107 aa, synthetic construct
DIQMTQSPSSLSASVGDRVTITCKASDHINNWLAWYQQKPGKVPKLLISGATSLETGVPSRFSGSGSGTDYTLTISSLQPEDVATYYCQQYWSTPYSFGGGTKLEIK

SEQ ID NO: 117 - protein, 107 aa, synthetic construct
DIQMTQSPSSLSASVGDRVTITCKASDHINNWLAWYQQKPGKVPKLLISGATSLETGVPSRFSGSGSGTDYTLTISSLQPEDVATYYCQQYGSTPYTFGGGTKLEIK

SEQ ID NO: 118 - protein, 107 aa, synthetic construct
DIQMTQSPSSLSASVGDRVTITCKASDHINNWLAWYQQKPGKVPKLLISGATSLETGVPSRFSGSGSGTDYTLTISSLQPEDVATYYCQQYWHTPYTFGGGTKLEIK

SEQ ID NO: 119 - protein, 17 aa, synthetic construct
YANPNNGASSYNQKFKG

SEQ ID NO: 120 - protein, 17 aa, synthetic construct
YINPNNGASSYNQKFKG

SEQ ID NO: 121 - protein, 17 aa, synthetic construct
YLNPNNGASSYNQKFKG

SEQ ID NO: 122 - protein, 17 aa, synthetic construct
YVNPNNGASNYNQKFKG

SEQ ID NO: 123 - protein, 17 aa, synthetic construct
YINPNNGASNYNQKFKG

SEQ ID NO: 124 - protein, 17 aa, synthetic construct
YLNPNNGATNYNQKFKG

SEQ ID NO: 125 - protein, 17 aa, synthetic construct
YANPNNGATNYNQKFKG

SEQ ID NO: 126 - protein, 12 aa, synthetic construct
WDGYVYYYGVDF

SEQ ID NO: 127 - protein, 12 aa, synthetic construct
WDGYSYYYGMDY

SEQ ID NO: 128 - protein, 12 aa, synthetic construct
WDGYVYYYGMDF

SEQ ID NO: 129 - protein, 12 aa, synthetic construct
WDGYSYYYGVDY

SEQ ID NO: 130 - protein, 12 aa, synthetic construct
WDGYSYYYGVDF

SEQ ID NO: 131 - protein, 12 aa, synthetic construct
WDGYSYYYGLDF

SEQ ID NO: 132 - protein, 11 aa, synthetic construct
KASEHVNNWLA

SEQ ID NO: 133 - protein, 11 aa, synthetic construct
KASEHINQWLA

SEQ ID NO: 134 - protein, 11 aa, synthetic construct
KASEHVNQWLA

SEQ ID NO: 135 - protein, 11 aa, synthetic construct
KASDHVNQWLA

SEQ ID NO: 136 - protein, 9 aa, synthetic construct
QQYWHTPYS

SEQ ID NO: 137 - protein, 9 aa, synthetic construct
QQYGSTPYS

SEQ ID NO: 138 - protein, 9 aa, synthetic construct
QQYGHTPYS

SEQ ID NO: 139 - protein, 9 aa, synthetic construct
QQYGHTPYT

SEQ ID NO: 140 - protein, 9 aa, synthetic construct
QQYWNTPYS

SEQ ID NO: 141 - protein, 9 aa, synthetic construct
QQYGNTPYS

SEQ ID NO: 142 - protein, 9 aa, synthetic construct
QQYGNTPYT

SEQ ID NO: 143 - protein, 453 aa, synthetic construct
QAYLQQSGAELVRSGASVKMSCKASGYTFTSYNIHWVKQTPGQGLEWIGYIYPGNGGTKYNERFKGKATLTADASSSTAYMQISSLTSEDSAVYFCARWRYYDRPTHYAMDYWGQGTSVTVSSASTKGPSVFPLAPSSKSTSGGTAALGCLVKDYFPEPVTVSWNSGALTSGVHTFPAVLQSSGLYSLSSVVTVPSSSLGTQTYICNVNHKPSNTKVDKKVEPKSCDKTHTCPPCPAPELLGGPSVFLFPPKPKDTLMISRTPEVTCVVVDVSHEDPEVKFNWYVDGVEVHNAKTKPREEQYNSTYRVVSVLTVLHQDWLNGKEYKCKVSNKALPAPIEKTISKAKGQPREPQVYTLPPSRDELTKNQVSLTCLVKGFYPSDIAVEWESNGQPENNYKTTPPVLDSDGSFFLYSKLTVDKSRWQQGNVFSCSVMHEALHNHYTQKSLSLSPGK

SEQ ID NO: 144 - protein, 450 aa, synthetic construct
EVQLVESGGDLVKPGGSLKLSCAASGFTFSSYGMSWVRQTPDKRLEWVATISSGGSYTYYPDSVKGRFTISRDNAKNTLYLQMSSLKSEDTAMYYCARPHYVSSYAMDYWGQGTSVTVSSASTKGPSVFPLAPSSKSTSGGTAALGCLVKDYFPEPVTVSWNSGALTSGVHTFPAVLQSSGLYSLSSVVTVPSSSLGTQTYICNVNHKPSNTKVDKKVEPKSCDKTHTCPPCPAPELLGGPSVFLFPPKPKDTLMISRTPEVTCVVVDVSHEDPEVKFNWYVDGVEVHNAKTKPREEQYNSTYRVVSVLTVLHQDWLNGKEYKCKVSNKALPAPIEKTISKAKGQPREPQVYTLPPSRDELTKNQVSLTCLVKGFYPSDIAVEWESNGQPENNYKTTPPVLDSDGSFFLYSKLTVDKSRWQQGNVFSCSVMHEALHNHYTQKSLSLSPGK

SEQ ID NO: 145 - protein, 451 aa, synthetic construct
EVQLVESGGGLVKPGGSLKLSCAASGFTFSNYAMSWVRQTPEKRLEWVATISDGGSYTSYPDNIKGRFTISRDNAKNNLYLQVTHLKSEDTAMYYCARDAILITTAGFAYWGQGTLLTVSAASTKGPSVFPLAPSSKSTSGGTAALGCLVKDYFPEPVTVSWNSGALTSGVHTFPAVLQSSGLYSLSSVVTVPSSSLGTQTYICNVNHKPSNTKVDKKVEPKSCDKTHTCPPCPAPELLGGPSVFLFPPKPKDTLMISRTPEVTCVVVDVSHEDPEVKFNWYVDGVEVHNAKTKPREEQYNSTYRVVSVLTVLHQDWLNGKEYKCKVSNKALPAPIEKTISKAKGQPREPQVYTLPPSRDELTKNQVSLTCLVKGFYPSDIAVEWESNGQPENNYKTTPPVLDSDGSFFLYSKLTVDKSRWQQGNVFSCSVMHEALHNHYTQKSLSLSPGK

SEQ ID NO: 146 - protein, 449 aa, synthetic construct
QGQLQQSGAELARPGASVKLSCKASGYTFTSYGISWVKQRTGQGLEWIGEIYPRSGNTYHNEKFKGKATLTADKSSSTAYMELRSLTSEDSAVYFCARSSYDYYAMDYWGQGTSVTVSSASTKGPSVFPLAPSSKSTSGGTAALGCLVKDYFPEPVTVSWNSGALTSGVHTFPAVLQSSGLYSLSSVVTVPSSSLGTQTYICNVNHKPSNTKVDKKVEPKSCDKTHTCPPCPAPELLGGPSVFLFPPKPKDTLMISRTPEVTCVVVDVSHEDPEVKFNWYVDGVEVHNAKTKPREEQYNSTYRVVSVLTVLHQDWLNGKEYKCKVSNKALPAPIEKTISKAKGQPREPQVYTLPPSRDELTKNQVSLTCLVKGFYPSDIAVEWESNGQPENNYKTTPPVLDSDGSFFLYSKLTVDKSRWQQGNVFSCSVMHEALHNHYTQKSLSLSPGK

SEQ ID NO: 147 - protein, 451 aa, synthetic construct
EVQLQQSGPELVKPGASVKMSCKASGYTFTDYNMHWVKKSHGKSLEWIGYINPNNGATNYNQKFKGKATLTVNKSSSTAYMELRSLTSEDSAVYNCARWDGYVYYYGMDYWGQGTSVTVSSASTKGPSVFPLAPSSKSTSGGTAALGCLVKDYFPEPVTVSWNSGALTSGVHTFPAVLQSSGLYSLSSVVTVPSSSLGTQTYICNVNHKPSNTKVDKKVEPKSCDKTHTCPPCPAPELLGGPSVFLFPPKPKDTLMISRTPEVTCVVVDVSHEDPEVKFNWYVDGVEVHNAKTKPREEQYNSTYRVVSVLTVLHQDWLNGKEYKCKVSNKALPAPIEKTISKAKGQPREPQVYTLPPSRDELTKNQVSLTCLVKGFYPSDIAVEWESNGQPENNYKTTPPVLDSDGSFFLYSKLTVDKSRWQQGNVFSCSVMHEALHNHYTQKSLSLSPGK

SEQ ID NO: 148 - protein, 453 aa, synthetic construct
QAYLQQSGAELVRSGASVKMSCKASGYTFTSYNMHWVKQTPGQGLEWIGYIYPGNGGTNYNQKFKGKATLTADTSSSTAYMQISSLTSEDSAVYFCARWKYYDKTTHYALDYWGQGTLVTVSSASTKGPSVFPLAPSSKSTSGGTAALGCLVKDYFPEPVTVSWNSGALTSGVHTFPAVLQSSGLYSLSSVVTVPSSSLGTQTYICNVNHKPSNTKVDKKVEPKSCDKTHTCPPCPAPELLGGPSVFLFPPKPKDTLMISRTPEVTCVVVDVSHEDPEVKFNWYVDGVEVHNAKTKPREEQYNSTYRVVSVLTVLHQDWLNGKEYKCKVSNKALPAPIEKTISKAKGQPREPQVYTLPPSRDELTKNQVSLTCLVKGFYPSDIAVEWESNGQPENNYKTTPPVLDSDGSFFLYSKLTVDKSRWQQGNVFSCSVMHEALHNHYTQKSLSLSPGK

SEQ ID NO: 149 - protein, 451 aa, synthetic construct
QVQLVQSGAEVKKPGASVKVSCKASGYTFTDYNMHWVRQAPGQGLEWIGYVNPNNGATSYNQKFKGRATMTRDTSTSTVYMELSSLRSEDTAVYYCARWDGYVYYYGLDYWGQGTLVTVSSASTKGPSVFPLAPSSKSTSGGTAALGCLVKDYFPEPVTVSWNSGALTSGVHTFPAVLQSSGLYSLSSVVTVPSSSLGTQTYICNVNHKPSNTKVDKKVEPKSCDKTHTCPPCPAPELLGGPSVFLFPPKPKDTLMISRTPEVTCVVVDVSHEDPEVKFNWYVDGVEVHNAKTKPREEQYNSTYRVVSVLTVLHQDWLNGKEYKCKVSNKALPAPIEKTISKAKGQPREPQVYTLPPSRDELTKNQVSLTCLVKGFYPSDIAVEWESNGQPENNYKTTPPVLDSDGSFFLYSKLTVDKSRWQQGNVFSCSVMHEALHNHYTQKSLSLSPGK

SEQ ID NO: 150 - protein, 451 aa, synthetic construct
QVQLVQSGAEVKKPGASVKVSCKASGYTFTDYNMHWVRQAPGQGLEWIGYVNPNNGATSYNQKFKGRVTMTVDTSTSTVYMELSSLRSEDTAVYNCARWDGYVYYYGLDYWGQGTLVTVSSASTKGPSVFPLAPSSKSTSGGTAALGCLVKDYFPEPVTVSWNSGALTSGVHTFPAVLQSSGLYSLSSVVTVPSSSLGTQTYICNVNHKPSNTKVDKKVEPKSCDKTHTCPPCPAPELLGGPSVFLFPPKPKDTLMISRTPEVTCVVVDVSHEDPEVKFNWYVDGVEVHNAKTKPREEQYNSTYRVVSVLTVLHQDWLNGKEYKCKVSNKALPAPIEKTISKAKGQPREPQVYTLPPSRDELTKNQVSLTCLVKGFYPSDIAVEWESNGQPENNYKTTPPVLDSDGSFFLYSKLTVDKSRWQQGNVFSCSVMHEALHNHYTQKSLSLSPGK

SEQ ID NO: 151 - protein, 451 aa, synthetic construct
QVQLVQSGAEVKKPGASVKVSCKASGYTFTDYNMHWVRQAPGQGLEWIGYVNPNNGATSYNQKFKGRATMTVDTSTSTVYMELSSLRSEDTAVYNCARWDGYVYYYGLDYWGQGTLVTVSSASTKGPSVFPLAPSSKSTSGGTAALGCLVKDYFPEPVTVSWNSGALTSGVHTFPAVLQSSGLYSLSSVVTVPSSSLGTQTYICNVNHKPSNTKVDKKVEPKSCDKTHTCPPCPAPELLGGPSVFLFPPKPKDTLMISRTPEVTCVVVDVSHEDPEVKFNWYVDGVEVHNAKTKPREEQYNSTYRVVSVLTVLHQDWLNGKEYKCKVSNKALPAPIEKTISKAKGQPREPQVYTLPPSRDELTKNQVSLTCLVKGFYPSDIAVEWESNGQPENNYKTTPPVLDSDGSFFLYSKLTVDKSRWQQGNVFSCSVMHEALHNHYTQKSLSLSPGK

SEQ ID NO: 152 - protein, 451 aa, synthetic construct
QVQLVQSGAEVKKPGASVKVSCKASGYTFTDYNMHWVRQAPGQSLEWIGYVNPNNGATSYNQKFKGRATMTVDKSTSTVYMELSSLRSEDTAVYNCARWDGYVYYYGLDYWGQGTLVTVSSASTKGPSVFPLAPSSKSTSGGTAALGCLVKDYFPEPVTVSWNSGALTSGVHTFPAVLQSSGLYSLSSVVTVPSSSLGTQTYICNVNHKPSNTKVDKKVEPKSCDKTHTCPPCPAPELLGGPSVFLFPPKPKDTLMISRTPEVTCVVVDVSHEDPEVKFNWYVDGVEVHNAKTKPREEQYNSTYRVVSVLTVLHQDWLNGKEYKCKVSNKALPAPIEKTISKAKGQPREPQVYTLPPSRDELTKNQVSLTCLVKGFYPSDIAVEWESNGQPENNYKTTPPVLDSDGSFFLYSKLTVDKSRWQQGNVFSCSVMHEALHNHYTQKSLSLSPGK

SEQ ID NO: 153 - protein, 451 aa, synthetic construct
QVQLVQSGAEVKKPGASVKVSCKASGYTFTDYNMHWVRQAPGQRLEWIGYINPNNGATNYNQKFKGRATITVDTSASTAYMELSSLRSEDTAVYYCARWDGYVYYYGMDYWGQGTLVTVSSASTKGPSVFPLAPSSKSTSGGTAALGCLVKDYFPEPVTVSWNSGALTSGVHTFPAVLQSSGLYSLSSVVTVPSSSLGTQTYICNVNHKPSNTKVDKKVEPKSCDKTHTCPPCPAPELLGGPSVFLFPPKPKDTLMISRTPEVTCVVVDVSHEDPEVKFNWYVDGVEVHNAKTKPREEQYNSTYRVVSVLTVLHQDWLNGKEYKCKVSNKALPAPIEKTISKAKGQPREPQVYTLPPSRDELTKNQVSLTCLVKGFYPSDIAVEWESNGQPENNYKTTPPVLDSDGSFFLYSKLTVDKSRWQQGNVFSCSVMHEALHNHYTQKSLSLSPGK

SEQ ID NO: 154 - protein, 451 aa, synthetic construct
QVQLVQSGAEVKKPGASVKVSCKASGYTFTDYNMHWVRQAPGQSLEWIGYINPNNGATNYNQKFKGRATITVDKSASTAYMELSSLRSEDTAVYNCARWDGYVYYYGMDYWGQGTLVTVSSASTKGPSVFPLAPSSKSTSGGTAALGCLVKDYFPEPVTVSWNSGALTSGVHTFPAVLQSSGLYSLSSVVTVPSSSLGTQTYICNVNHKPSNTKVDKKVEPKSCDKTHTCPPCPAPELLGGPSVFLFPPKPKDTLMISRTPEVTCVVVDVSHEDPEVKFNWYVDGVEVHNAKTKPREEQYNSTYRVVSVLTVLHQDWLNGKEYKCKVSNKALPAPIEKTISKAKGQPREPQVYTLPPSRDELTKNQVSLTCLVKGFYPSDIAVEWESNGQPENNYKTTPPVLDSDGSFFLYSKLTVDKSRWQQGNVFSCSVMHEALHNHYTQKSLSLSPGK

SEQ ID NO: 155 - protein, 451 aa, synthetic construct
QVQLVQSGAEVKKPGASVKVSCKASGYTFTDYNMHWVRQAPGQRLEWIGYINPNNGATNYNQKFKGRVTITVDTSASTAYMELSSLRSEDTAVYNCARWDGYVYYYGMDYWGQGTLVTVSSASTKGPSVFPLAPSSKSTSGGTAALGCLVKDYFPEPVTVSWNSGALTSGVHTFPAVLQSSGLYSLSSVVTVPSSSLGTQTYICNVNHKPSNTKVDKKVEPKSCDKTHTCPPCPAPELLGGPSVFLFPPKPKDTLMISRTPEVTCVVVDVSHEDPEVKFNWYVDGVEVHNAKTKPREEQYNSTYRVVSVLTVLHQDWLNGKEYKCKVSNKALPAPIEKTISKAKGQPREPQVYTLPPSRDELTKNQVSLTCLVKGFYPSDIAVEWESNGQPENNYKTTPPVLDSDGSFFLYSKLTVDKSRWQQGNVFSCSVMHEALHNHYTQKSLSLSPGK

SEQ ID NO: 156 - protein, 451 aa, synthetic construct
QVQLVQSGAEVKKPGASVKVSCKASGYTFTDYNMHWVRQAPGQSLEWIGYINPNNGATNYNQKFKGRATITVDTSASTAYMELSSLRSEDTAVYNCARWDGYVYYYGMDYWGQGTLVTVSSASTKGPSVFPLAPSSKSTSGGTAALGCLVKDYFPEPVTVSWNSGALTSGVHTFPAVLQSSGLYSLSSVVTVPSSSLGTQTYICNVNHKPSNTKVDKKVEPKSCDKTHTCPPCPAPELLGGPSVFLFPPKPKDTLMISRTPEVTCVVVDVSHEDPEVKFNWYVDGVEVHNAKTKPREEQYNSTYRVVSVLTVLHQDWLNGKEYKCKVSNKALPAPIEKTISKAKGQPREPQVYTLPPSRDELTKNQVSLTCLVKGFYPSDIAVEWESNGQPENNYKTTPPVLDSDGSFFLYSKLTVDKSRWQQGNVFSCSVMHEALHNHYTQKSLSLSPGK

SEQ ID NO: 157 - protein, 451 aa, synthetic construct
QVQLVQSGAEVKKPGASVKVSCKASGYTFTDYNMHWVRQATGQGLEWIGYINPNNGATNYNQKFKGRATMTRNKSISTAYMELRSLRSEDTAVYYCARWDGYVYYYGMDYWGQGTLVTVSSASTKGPSVFPLAPSSKSTSGGTAALGCLVKDYFPEPVTVSWNSGALTSGVHTFPAVLQSSGLYSLSSVVTVPSSSLGTQTYICNVNHKPSNTKVDKKVEPKSCDKTHTCPPCPAPELLGGPSVFLFPPKPKDTLMISRTPEVTCVVVDVSHEDPEVKFNWYVDGVEVHNAKTKPREEQYNSTYRVVSVLTVLHQDWLNGKEYKCKVSNKALPAPIEKTISKAKGQPREPQVYTLPPSRDELTKNQVSLTCLVKGFYPSDIAVEWESNGQPENNYKTTPPVLDSDGSFFLYSKLTVDKSRWQQGNVFSCSVMHEALHNHYTQKSLSLSPGK

SEQ ID NO: 158 - protein, 451 aa, synthetic construct
QVQLVQSGAEVKKPGASVKVSCKASGYTFTDYNMHWVRQATGQGLEWIGYINPNNGATNYNQKFKGRATMTRNKSISTAYMELRSLRSEDTAVYNCARWDGYVYYYGMDYWGQGTLVTVSSASTKGPSVFPLAPSSKSTSGGTAALGCLVKDYFPEPVTVSWNSGALTSGVHTFPAVLQSSGLYSLSSVVTVPSSSLGTQTYICNVNHKPSNTKVDKKVEPKSCDKTHTCPPCPAPELLGGPSVFLFPPKPKDTLMISRTPEVTCVVVDVSHEDPEVKFNWYVDGVEVHNAKTKPREEQYNSTYRVVSVLTVLHQDWLNGKEYKCKVSNKALPAPIEKTISKAKGQPREPQVYTLPPSRDELTKNQVSLTCLVKGFYPSDIAVEWESNGQPENNYKTTPPVLDSDGSFFLYSKLTVDKSRWQQGNVFSCSVMHEALHNHYTQKSLSLSPGK

SEQ ID NO: 159 - protein, 451 aa, synthetic construct
QVQLVQSGAEVKKPGASVKVSCKASGYTFTDYNMHWVRQATGQGLEWIGYINPNNGATNYNQKFKGRATLTVNKSISTAYMELRSLRSEDTAVYYCARWDGYVYYYGMDYWGQGTLVTVSSASTKGPSVFPLAPSSKSTSGGTAALGCLVKDYFPEPVTVSWNSGALTSGVHTFPAVLQSSGLYSLSSVVTVPSSSLGTQTYICNVNHKPSNTKVDKKVEPKSCDKTHTCPPCPAPELLGGPSVFLFPPKPKDTLMISRTPEVTCVVVDVSHEDPEVKFNWYVDGVEVHNAKTKPREEQYNSTYRVVSVLTVLHQDWLNGKEYKCKVSNKALPAPIEKTISKAKGQPREPQVYTLPPSRDELTKNQVSLTCLVKGFYPSDIAVEWESNGQPENNYKTTPPVLDSDGSFFLYSKLTVDKSRWQQGNVFSCSVMHEALHNHYTQKSLSLSPGK

SEQ ID NO: 160 - protein, 451 aa, synthetic construct
QVQLVQSGAEVKKPGASVKVSCKASGYTFTDYNMHWVRKATGQSLEWIGYINPNNGATNYNQKFKGRATMTRNKSISTAYMELRSLRSEDTAVYNCARWDGYVYYYGMDYWGQGTLVTVSSASTKGPSVFPLAPSSKSTSGGTAALGCLVKDYFPEPVTVSWNSGALTSGVHTFPAVLQSSGLYSLSSVVTVPSSSLGTQTYICNVNHKPSNTKVDKKVEPKSCDKTHTCPPCPAPELLGGPSVFLFPPKPKDTLMISRTPEVTCVVVDVSHEDPEVKFNWYVDGVEVHNAKTKPREEQYNSTYRVVSVLTVLHQDWLNGKEYKCKVSNKALPAPIEKTISKAKGQPREPQVYTLPPSRDELTKNQVSLTCLVKGFYPSDIAVEWESNGQPENNYKTTPPVLDSDGSFFLYSKLTVDKSRWQQGNVFSCSVMHEALHNHYTQKSLSLSPGK

SEQ ID NO: 161 - protein, 453 aa, synthetic construct
QAYLQQSGAELVRSGASVKMSCKASGYTFTSYNMHWVKQTPGQGLEWIGYIYPGNAGTNYNQKFKGKATLTADTSSSTAYMQISSLTSEDSAVYFCARWKYYDKTTHYALDYWGQGTLVTVSSASTKGPSVFPLAPSSKSTSGGTAALGCLVKDYFPEPVTVSWNSGALTSGVHTFPAVLQSSGLYSLSSVVTVPSSSLGTQTYICNVNHKPSNTKVDKKVEPKSCDKTHTCPPCPAPELLGGPSVFLFPPKPKDTLMISRTPEVTCVVVDVSHEDPEVKFNWYVDGVEVHNAKTKPREEQYNSTYRVVSVLTVLHQDWLNGKEYKCKVSNKALPAPIEKTISKAKGQPREPQVYTLPPSRDELTKNQVSLTCLVKGFYPSDIAVEWESNGQPENNYKTTPPVLDSDGSFFLYSKLTVDKSRWQQGNVFSCSVMHEALHNHYTQKSLSLSPGK

SEQ ID NO: 162 - protein, 453 aa, synthetic construct
QAYLQQSGAELVRSGASVKMSCKASGYTFTSYNMHWVKQTPGQGLEWIGYIYPGNQGTNYNQKFKGKATLTADTSSSTAYMQISSLTSEDSAVYFCARWKYYDKTTHYALDYWGQGTLVTVSSASTKGPSVFPLAPSSKSTSGGTAALGCLVKDYFPEPVTVSWNSGALTSGVHTFPAVLQSSGLYSLSSVVTVPSSSLGTQTYICNVNHKPSNTKVDKKVEPKSCDKTHTCPPCPAPELLGGPSVFLFPPKPKDTLMISRTPEVTCVVVDVSHEDPEVKFNWYVDGVEVHNAKTKPREEQYNSTYRVVSVLTVLHQDWLNGKEYKCKVSNKALPAPIEKTISKAKGQPREPQVYTLPPSRDELTKNQVSLTCLVKGFYPSDIAVEWESNGQPENNYKTTPPVLDSDGSFFLYSKLTVDKSRWQQGNVFSCSVMHEALHNHYTQKSLSLSPGK

SEQ ID NO: 163 - protein, 451 aa, synthetic construct
EVQLQQSGPELVKPGASVKMSCKASGYTFTDYNMHWVKKSHGKSLEWIGYVNPNNAATSYNQKFKGKATLTVNKSSSTAYMELRSLTSEDSAVYNCARWDGYVYYYGLDYWGQGTSVTVSSASTKGPSVFPLAPSSKSTSGGTAALGCLVKDYFPEPVTVSWNSGALTSGVHTFPAVLQSSGLYSLSSVVTVPSSSLGTQTYICNVNHKPSNTKVDKKVEPKSCDKTHTCPPCPAPELLGGPSVFLFPPKPKDTLMISRTPEVTCVVVDVSHEDPEVKFNWYVDGVEVHNAKTKPREEQYNSTYRVVSVLTVLHQDWLNGKEYKCKVSNKALPAPIEKTISKAKGQPREPQVYTLPPSRDELTKNQVSLTCLVKGFYPSDIAVEWESNGQPENNYKTTPPVLDSDGSFFLYSKLTVDKSRWQQGNVFSCSVMHEALHNHYTQKSLSLSPGK

SEQ ID NO: 164 - protein, 451 aa, synthetic construct
EVQLQQSGPELVKPGASVKMSCKASGYTFTDYNMHWVKKSHGKSLEWIGYVNPNQGATSYNQKFKGKATLTVNKSSSTAYMELRSLTSEDSAVYNCARWDGYVYYYGLDYWGQGTSVTVSSASTKGPSVFPLAPSSKSTSGGTAALGCLVKDYFPEPVTVSWNSGALTSGVHTFPAVLQSSGLYSLSSVVTVPSSSLGTQTYICNVNHKPSNTKVDKKVEPKSCDKTHTCPPCPAPELLGGPSVFLFPPKPKDTLMISRTPEVTCVVVDVSHEDPEVKFNWYVDGVEVHNAKTKPREEQYNSTYRVVSVLTVLHQDWLNGKEYKCKVSNKALPAPIEKTISKAKGQPREPQVYTLPPSRDELTKNQVSLTCLVKGFYPSDIAVEWESNGQPENNYKTTPPVLDSDGSFFLYSKLTVDKSRWQQGNVFSCSVMHEALHNHYTQKSLSLSPGK

SEQ ID NO: 165 - protein, 451 aa, synthetic construct
EVQLQQSGPELVKPGASVKMSCKASGYTFTDYNMHWVKKSHGKSLEWIGYVNPNNGATSYNQKFKGKATLTVNKSSSTAYMELRSLTSEDSAVYNCARWDAYVYYYGLDYWGQGTSVTVSSASTKGPSVFPLAPSSKSTSGGTAALGCLVKDYFPEPVTVSWNSGALTSGVHTFPAVLQSSGLYSLSSVVTVPSSSLGTQTYICNVNHKPSNTKVDKKVEPKSCDKTHTCPPCPAPELLGGPSVFLFPPKPKDTLMISRTPEVTCVVVDVSHEDPEVKFNWYVDGVEVHNAKTKPREEQYNSTYRVVSVLTVLHQDWLNGKEYKCKVSNKALPAPIEKTISKAKGQPREPQVYTLPPSRDELTKNQVSLTCLVKGFYPSDIAVEWESNGQPENNYKTTPPVLDSDGSFFLYSKLTVDKSRWQQGNVFSCSVMHEALHNHYTQKSLSLSPGK

SEQ ID NO: 166 - protein, 451 aa, synthetic construct
EVQLQQSGPELVKPGASVKMSCKASGYTFTDYNMHWVKKSHGKSLEWIGYVNPNNGATSYNQKFKGKATLTVNKSSSTAYMELRSLTSEDSAVYNCARWEGYVYYYGLDYWGQGTSVTVSSASTKGPSVFPLAPSSKSTSGGTAALGCLVKDYFPEPVTVSWNSGALTSGVHTFPAVLQSSGLYSLSSVVTVPSSSLGTQTYICNVNHKPSNTKVDKKVEPKSCDKTHTCPPCPAPELLGGPSVFLFPPKPKDTLMISRTPEVTCVVVDVSHEDPEVKFNWYVDGVEVHNAKTKPREEQYNSTYRVVSVLTVLHQDWLNGKEYKCKVSNKALPAPIEKTISKAKGQPREPQVYTLPPSRDELTKNQVSLTCLVKGFYPSDIAVEWESNGQPENNYKTTPPVLDSDGSFFLYSKLTVDKSRWQQGNVFSCSVMHEALHNHYTQKSLSLSPGK

SEQ ID NO: 167 - protein, 451 aa, synthetic construct
QVQLVQSGAEVKKPGASVKVSCKASGYTFTDYNMHWVRQAPGQSLEWIGYVNPNNAATSYNQKFKGRATMTVDKSTSTVYMELSSLRSEDTAVYNCARWDGYVYYYGLDYWGQGTLVTVSSASTKGPSVFPLAPSSKSTSGGTAALGCLVKDYFPEPVTVSWNSGALTSGVHTFPAVLQSSGLYSLSSVVTVPSSSLGTQTYICNVNHKPSNTKVDKKVEPKSCDKTHTCPPCPAPELLGGPSVFLFPPKPKDTLMISRTPEVTCVVVDVSHEDPEVKFNWYVDGVEVHNAKTKPREEQYNSTYRVVSVLTVLHQDWLNGKEYKCKVSNKALPAPIEKTISKAKGQPREPQVYTLPPSRDELTKNQVSLTCLVKGFYPSDIAVEWESNGQPENNYKTTPPVLDSDGSFFLYSKLTVDKSRWQQGNVFSCSVMHEALHNHYTQKSLSLSPGK

SEQ ID NO: 168 - protein, 218 aa, synthetic construct
DIVVTQSPASLAVSLGQRATISCRASKSVSTSGFSYLHWFQQKPGQPPKLLIYLASNLESGVPARFSGSGSGTDFTLNIHPVEEEDVAVYYCQHSREFPFTFGSGTKLEIKRTVAAPSVFIFPPSDEQLKSGTASVVCLLNNFYPREAKVQWKVDNALQSGNSQESVTEQDSKDSTYSLSSTLTLSKADYEKHKVYACEVTHQGLSSPVTKSFNRGEC

SEQ ID NO: 169 - protein, 214 aa, synthetic construct
DIQMTQSSSSFSVSLGDRVTITCKASEDIYNRLAWYQQKPGNAPRLLISGATSLETGVPSRFSGSGSGKDYTLSITSLQTEDVATYYCQQYWSTPPTFGGGTKLEIKRTVAAPSVFIFPPSDEQLKSGTASVVCLLNNFYPREAKVQWKVDNALQSGNSQESVTEQDSKDSTYSLSSTLTLSKADYEKHKVYACEVTHQGLSSPVTKSFNRGEC

SEQ ID NO: 170 - protein, 214 aa, synthetic construct
DIQMTQSSSSFSVSLGDRVTITCKASEDIYNRLAWYQQKPGNAPRLLISATTSLETGVPSRFSGSGSGKDYTLSITSLQTEDVATYYCQQYWSFPRTFGGGTKLEVKRTVAAPSVFIFPPSDEQLKSGTASVVCLLNNFYPREAKVQWKVDNALQSGNSQESVTEQDSKDSTYSLSSTLTLSKADYEKHKVYACEVTHQGLSSPVTKSFNRGEC

SEQ ID NO: 171 - protein, 215 aa, synthetic construct
EIVVTQSPALMAASPGEKVTITCSVSSIISSSKLHWYQQKSETSPKPWIYGTSNLASGVPIRFSGSGSGTSYSLTISSMEAEDAATYYCQQWSSYPLTFGAGTKLELKRTVAAPSVFIFPPSDEQLKSGTASVVCLLNNFYPREAKVQWKVDNALQSGNSQESVTEQDSKDSTYSLSSTLTLSKADYEKHKVYACEVTHQGLSSPVTKSFNRGEC

SEQ ID NO: 172 - protein, 214 aa, synthetic construct
DIQMTQSSSYLSVSLGGRVTITCKASDHINNWLAWYQQKPGNAPRLLISGATSLETGVPSRFSGSGSGKDYTLSITSLQTEDVATYYCQQYWNTPYTFGGGTKLEIKRTVAAPSVFIFPPSDEQLKSGTASVVCLLNNFYPREAKVQWKVDNALQSGNSQESVTEQDSKDSTYSLSSTLTLSKADYEKHKVYACEVTHQGLSSPVTKSFNRGEC

SEQ ID NO: 173 - protein, 218 aa, synthetic construct
DIVLTQSPASLAVSLGQWATISCRASKSVSTSGYSYIHWHQQKPGQPPKLLIYLASNLESGVPARFSGSGSGTDFTLNIHPVEEEDAATYYCHHSRELPFTFGSGTKLEIKRTVAAPSVFIFPPSDEQLKSGTASVVCLLNNFYPREAKVQWKVDNALQSGNSQESVTEQDSKDSTYSLSSTLTLSKADYEKHKVYACEVTHQGLSSPVTKSFNRGEC

SEQ ID NO: 174 - protein, 214 aa, synthetic construct
DIQMTQSPSSLSASVGDRVTITCKASDHINNWLAWYQQKPGKVPKLLISGATSLETGVPSRFSGSGSGTDYTLTISSLQPEDVATYYCQQYWSTPYTFGGGTKLEIKRTVAAPSVFIFPPSDEQLKSGTASVVCLLNNFYPREAKVQWKVDNALQSGNSQESVTEQDSKDSTYSLSSTLTLSKADYEKHKVYACEVTHQGLSSPVTKSFNRGEC

SEQ ID NO: 175 - protein, 214 aa, synthetic construct
DIQMTQSPSSLSASVGGRVTITCKASDHINNWLAWYQQKPGKVPRLLISGATSLETGVPSRFSGSGSGTDYTLTISSLQPEDVATYYCQQYWSTPYTFGGGTKLEIKRTVAAPSVFIFPPSDEQLKSGTASVVCLLNNFYPREAKVQWKVDNALQSGNSQESVTEQDSKDSTYSLSSTLTLSKADYEKHKVYACEVTHQGLSSPVTKSFNRGEC

SEQ ID NO: 176 - protein, 214 aa, synthetic construct
DIQMTQSPSSLSASVGDRVTITCKASDHINNWLAWYQQKPGKAPKLLISGATSLETGVPSRFSGSGSGTDYTFTISSLQPEDIATYYCQQYWNTPYTFGGGTKLEIKRTVAAPSVFIFPPSDEQLKSGTASVVCLLNNFYPREAKVQWKVDNALQSGNSQESVTEQDSKDSTYSLSSTLTLSKADYEKHKVYACEVTHQGLSSPVTKSFNRGEC

SEQ ID NO: 177 - protein, 214 aa, synthetic construct
DIQMTQSPSSLSASVGGRVTITCKASDHINNWLAWYQQKPGKAPKLLISGATSLETGVPSRFSGSGSGTDYTFTISSLQPEDIATYYCQQYWNTPYTFGGGTKLEIKRTVAAPSVFIFPPSDEQLKSGTASVVCLLNNFYPREAKVQWKVDNALQSGNSQESVTEQDSKDSTYSLSSTLTLSKADYEKHKVYACEVTHQGLSSPVTKSFNRGEC

SEQ ID NO: 178 - protein, 214 aa, synthetic construct
DIQMTQSPSSLSASVGDRVTITCKASDHINNWLAWYQQKPGKVPRLLISGATSLETGVPSRFSGSGSGKDYTLTISSLQPEDVATYYCQQYWNTPYTFGGGTKLEIKRTVAAPSVFIFPPSDEQLKSGTASVVCLLNNFYPREAKVQWKVDNALQSGNSQESVTEQDSKDSTYSLSSTLTLSKADYEKHKVYACEVTHQGLSSPVTKSFNRGEC

SEQ ID NO: 179 - protein, 9 aa, synthetic construct
QQWSSYPLT